European Patent Application EP 4 714 979 A1, published March 25, 2026. Title: 偏向性补体抑制杂合蛋白. Applicant: 天辰生物医药（苏州）有限公司. The sequence listing filed with the application follows.

SEQUENCE LISTING (41 sequences)

SEQ ID NO: 1 - protein, 381 aa, synthetic construct
MTVARPSVPAALPLLGELPRLLLLVLLCLPAVWGDCGLPPDVPNAQPALEGRTSFPEDTVITYKCEESFVKIPGEKDSVICLKGSQWSDIEEFCNRSCEVPTRLNSASLKQPYITQNYFPVGTVVEYECRPGYRREPSLSPKLTCLQNLKWSTAVEFCKKKSCPNPGEIRNGQIDVPGGILFGATISFSCNTGYKLFGSTSSFCLISGSSVQWSDPLPECREIYCPAPPQIDNGIIQGERDHYGYRQSVTYACNKGFTMIGEHSIYCTVNNDEGEWSGPPPECRGKSLTSKVPPTVQKPTTVNVPTTEVSPTSQKTTTKTTTPNAQATRSTPVSRTTKHFHETTPNKGSGTTSGTTRLLSGHTCFTLTGLLGTLVTMGLLT

SEQ ID NO: 2 - DNA, 1146 bp, synthetic construct
  source 1..1146: mol_type = other DNA
atgaccgtcgcgcggccgagcgtgcccgcggcgctgcccctcctcggggagctgccccggctgctgctgctggtgctgttgtgcctgccggccgtgtggggtgactgtggccttcccccagatgtacctaatgcccagccagctttggaaggccgtacaagttttcccgaggatactgtaataacgtacaaatgtgaagaaagctttgtgaaaattcctggcgagaaggactcagtgatctgccttaagggcagtcaatggtcagatattgaagagttctgcaatcgtagctgcgaggtgccaacaaggctaaattctgcatccctcaaacagccttatatcactcagaattattttccagtcggtactgttgtggaatatgagtgccgtccaggttacagaagagaaccttctctatcaccaaaactaacttgccttcagaatttaaaatggtccacagcagtcgaattttgtaaaaagaaatcatgccctaatccgggagaaatacgaaatggtcagattgatgtaccaggtggcatattatttggtgcaaccatctccttctcatgtaacacagggtacaaattatttggctcgacttctagtttttgtcttatttcaggcagctctgtccagtggagtgacccgttgccagagtgcagagaaatttattgtccagcaccaccacaaattgacaatggaataattcaaggggaacgtgaccattatggatatagacagtctgtaacgtatgcatgtaataaaggattcaccatgattggagagcactctatttattgtactgtgaataatgatgaaggagagtggagtggcccaccacctgaatgcagaggaaaatctctaacttccaaggtcccaccaacagttcagaaacctaccacagtaaatgttccaactacagaagtctcaccaacttctcagaaaaccaccacaaaaaccaccacaccaaatgctcaagcaacacggagtacacctgtttccaggacaaccaagcattttcatgaaacaaccccaaataaaggaagtggaaccacttcaggtactacccgtcttctatctgggcacacgtgtttcacgttgacaggtttgcttgggacgctagtaaccatgggcttgctgacttag

SEQ ID NO: 3 - protein, 1231 aa, synthetic construct
MRLLAKIICLMLWAICVAEDCNELPPRRNTEILTGSWSDQTYPEGTQAIYKCRPGYRSLGNVIMVCRKGEWVALNPLRKCQKRPCGHPGDTPFGTFTLTGGNVFEYGVKAVYTCNEGYQLLGEINYRECDTDGWTNDIPICEVVKCLPVTAPENGKIVSSAMEPDREYHFGQAVRFVCNSGYKIEGDEEMHCSDDGFWSKEKPKCVEISCKSPDVINGSPISQKIIYKENERFQYKCNMGYEYSERGDAVCTESGWRPLPSCEEKSCDNPYIPNGDYSPLRIKHRTGDEITYQCRNGFYPATRGNTAKCTSTGWIPAPRCTLKPCDYPDIKHGGLYHENMRRPYFPVAVGKYYSYYCDEHFETPSGSYWDHIHCTQDGWSPAVPCLRKCYFPYLENGYNQNYGRKFVQGKSIDVACHPGYALPKAQTTVTCMENGWSPTPRCIRVKTCSKSSIDIENGFISESQYTYALKEKAKYQCKLGYVTADGETSGSITCGKDGWSAQPTCIKSCDIPVFMNARTKNDFTWFKLNDTLDYECHDGYESNTGSTTGSIVCGYNGWSDLPICYERECELPKIDVHLVPDRKKDQYKVGEVLKFSCKPGFTIVGPNSVQCYHFGLSPDLPICKEQVQSCGPPPELLNGNVKEKTKEEYGHSEVVEYYCNPRFLMKGPNKIQCVDGEWTTLPVCIVEESTCGDIPELEHGWAQLSSPPYYYGDSVEFNCSESFTMIGHRSITCIHGVWTQLPQCVAIDKLKKCKSSNLIILEEHLKNKKEFDHNSNIRYRCRGKEGWIHTVCINGRWDPEVNCSMAQIQLCPPPPQIPNSHNMTTTLNYRDGEKVSVLCQENYLIQEGEEITCKDGRWQSIPLCVEKIPCSQPPQIEHGTINSSRSSQESYAHGTKLSYTCEGGFRISEENETTCYMGKWSSPPQCEGLPCKSPPEISHGVVAHMSDSYQYGEEVTYKCFEGFGIDGPAIAKCLGEKWSHPPSCIKTDCLSLPSFENAIPMGEKKDVYKAGEQVTYTCATYYKMDGASNVTCINSRWTGRPTCRDTSCVNPPTVQNAYIVSRQMSKYPSGERVRYQCRSPYEMFGDEEVMCLNGNWTEPPQCKDSTGKCGPPPPIDNGDITSFPLSVYAPASSVEYQCQNLYQLEGNKRITCRNGQWSEPPKCLHPCVISREIMENYNIALRWTAKQKLYSRTGESVEFVCKRGYRLSSRSHTLRTTCWDGKLEYPTCAKR

SEQ ID NO: 4 - DNA, 3696 bp, synthetic construct
  source 1..3696: mol_type = other DNA
atgagacttctagcaaagattatttgccttatgttatgggctatttgtgtagcagaagattgcaatgaacttcctccaagaagaaatacagaaattctgacaggttcctggtctgaccaaacatatccagaaggcacccaggctatctataaatgccgccctggatatagatctcttggaaatgtaataatggtatgcaggaagggagaatgggttgctcttaatccattaaggaaatgtcagaaaaggccctgtggacatcctggagatactccttttggtacttttacccttacaggaggaaatgtgtttgaatatggtgtaaaagctgtgtatacatgtaatgaggggtatcaattgctaggtgagattaattaccgtgaatgtgacacagatggatggaccaatgatattcctatatgtgaagttgtgaagtgtttaccagtgacagcaccagagaatggaaaaattgtcagtagtgcaatggaaccagatcgggaataccattttggacaagcagtacggtttgtatgtaactcaggctacaagattgaaggagatgaagaaatgcattgttcagacgatggtttttggagtaaagagaaaccaaagtgtgtggaaatttcatgcaaatccccagatgttataaatggatctcctatatctcagaagattatttataaggagaatgaacgatttcaatataaatgtaacatgggttatgaatacagtgaaagaggagatgctgtatgcactgaatctggatggcgtccgttgccttcatgtgaagaaaaatcatgtgataatccttatattccaaatggtgactactcacctttaaggattaaacacagaactggagatgaaatcacgtaccagtgtagaaatggtttttatcctgcaacccggggaaatacagcaaaatgcacaagtactggctggatacctgctccgagatgtaccttgaaaccttgtgattatccagacattaaacatggaggtctatatcatgagaatatgcgtagaccatactttccagtagctgtaggaaaatattactcctattactgtgatgaacattttgagactccgtcaggaagttactgggatcacattcattgcacacaagatggatggtcgccagcagtaccatgcctcagaaaatgttattttccttatttggaaaatggatataatcaaaatcatggaagaaagtttgtacagggtaaatctatagacgttgcctgccatcctggctacgctcttccaaaagcgcagaccacagttacatgtatggagaatggctggtctcctactcccagatgcatccgtgtcaaaacatgttccaaatcaagtatagatattgagaatgggtttatttctgaatctcagtatacatatgccttaaaagaaaaagcgaaatatcaatgcaaactaggatatgtaacagcagatggtgaaacatcaggatcaattacatgtgggaaagatggatggtcagctcaacccacgtgcattaaatcttgtgatatcccagtatttatgaatgccagaactaaaaatgacttcacatggtttaagctgaatgacacattggactatgaatgccatgatggttatgaaagcaatactggaagcaccactggttccatagtgtgtggttacaatggttggtctgatttacccatatgttatgaaagagaatgcgaacttcctaaaatagatgtacacttagttcctgatcgcaagaaagaccagtataaagttggagaggtgttgaaattctcctgcaaaccaggatttacaatagttggacctaattccgttcagtgctaccactttggattgtctcctgacctcccaatatgtaaagagcaagtacaatcatgtggtccacctcctgaactcctcaatgggaatgttaaggaaaaaacgaaagaagaatatggacacagtgaagtggtggaatattattgcaatcctagatttctaatgaagggacctaataaaattcaatgtgttgatggagagtggacaactttaccagtgtgtattgtggaggagagtacctgtggagatatacctgaacttgaacatggctgggcccagctttcttcccctccttattactatggagattcagtggaattcaattgctcagaatcatttacaatgattggacacagatcaattacgtgtattcatggagtatggacccaacttccccagtgtgtggcaatagataaacttaagaagtgcaaatcatcaaatttaattatacttgaggaacatttaaaaaacaagaaggaattcgatcataattctaacataaggtacagatgtagaggaaaagaaggatggatacacacagtctgcataaatggaagatgggatccagaagtgaactgctcaatggcacaaatacaattatgcccacctccacctcagattcccaattctcacaatatgacaaccacactgaattatcgggatggagaaaaagtatctgttctttgccaagaaaattatctaattcaggaaggagaagaaattacatgcaaagatggaagatggcagtcaataccactctgtgttgaaaaaattccatgttcacaaccacctcagatagaacacggaaccattaattcatccaggtcttcacaagaaagttatgcacatgggactaaattgagttatacttgtgagggtggtttcaggatatctgaagaaaatgaaacaacatgctacatgggaaaatggagttctccacctcagtgtgaaggccttccttgtaaatctccacctgagatttctcatggtgttgtagctcacatgtcagacagttatcagtatggagaagaagttacgtacaaatgttttgaaggttttggaattgatgggcctgcaattgcaaaatgcttaggagaaaaatggtctcaccctccatcatgcataaaaacagattgtctcagtttacctagctttgaaaatgccatacccatgggagagaagaaggatgtgtataaggcgggtgagcaagtgacttacacttgtgcaacatattacaaaatggatggagccagtaatgtaacatgcattaatagcagatggacaggaaggccaacatgcagagacacctcctgtgtgaatccgcccacagtacaaaatgcttatatagtgtcgagacagatgagtaaatatccatctggtgagagagtacgttatcaatgtaggagcccttatgaaatgtttggggatgaagaagtgatgtgtttaaatggaaactggacggaaccacctcaatgcaaagattctacaggaaaatgtgggccccctccacctattgacaatggggacattacttcattcccgttgtcagtatatgctccagcttcatcagttgagtaccaatgccagaacttgtatcaacttgagggtaacaagcgaataacatgtagaaatggacaatggtcagaaccaccaaaatgcttacatccgtgtgtaatatcccgagaaattatggaaaattataacatagcattaaggtggacagccaaacagaagctttattcgagaacaggtgaatcagttgaatttgtgtgtaaacggggatatcgtctttcatcacgttctcacacattgcgaacaacatgttgggatgggaaactggagtatccaacttgtgcaaaaagatag

SEQ ID NO: 5 - protein, 449 aa, synthetic construct
MRLLAKIICLMLWAICVAEDCNELPPRRNTEILTGSWSDQTYPEGTQAIYKCRPGYRSLGNVIMVCRKGEWVALNPLRKCQKRPCGHPGDTPFGTFTLTGGNVFEYGVKAVYTCNEGYQLLGEINYRECDTDGWTNDIPICEVVKCLPVTAPENGKIVSSAMEPDREYHFGQAVRFVCNSGYKIEGDEEMHCSDDGFWSKEKPKCVEISCKSPDVINGSPISQKIIYKENERFQYKCNMGYEYSERGDAVCTESGWRPLPSCEEKSCDNPYIPNGDYSPLRIKHRTGDEITYQCRNGFYPATRGNTAKCTSTGWIPAPRCTLKPCDYPDIKHGGLYHENMRRPYFPVAVGKYYSYYCDEHFETPSGSYWDHIHCTQDGWSPAVPCLRKCYFPYLENGYNQNYGRKFVQGKSIDVACHPGYALPKAQTTVTCMENGWSPTPRCIRVSFTL

SEQ ID NO: 6 - DNA, 1350 bp, synthetic construct
  source 1..1350: mol_type = other DNA
atgagacttctagcaaagattatttgccttatgttatgggctatttgtgtagcagaagattgcaatgaacttcctccaagaagaaatacagaaattctgacaggttcctggtctgaccaaacatatccagaaggcacccaggctatctataaatgccgccctggatatagatctcttggaaatgtaataatggtatgcaggaagggagaatgggttgctcttaatccattaaggaaatgtcagaaaaggccctgtggacatcctggagatactccttttggtacttttacccttacaggaggaaatgtgtttgaatatggtgtaaaagctgtgtatacatgtaatgaggggtatcaattgctaggtgagattaattaccgtgaatgtgacacagatggatggaccaatgatattcctatatgtgaagttgtgaagtgtttaccagtgacagcaccagagaatggaaaaattgtcagtagtgcaatggaaccagatcgggaataccattttggacaagcagtacggtttgtatgtaactcaggctacaagattgaaggagatgaagaaatgcattgttcagacgatggtttttggagtaaagagaaaccaaagtgtgtggaaatttcatgcaaatccccagatgttataaatggatctcctatatctcagaagattatttataaggagaatgaacgatttcaatataaatgtaacatgggttatgaatacagtgaaagaggagatgctgtatgcactgaatctggatggcgtccgttgccttcatgtgaagaaaaatcatgtgataatccttatattccaaatggtgactactcacctttaaggattaaacacagaactggagatgaaatcacgtaccagtgtagaaatggtttttatcctgcaacccggggaaatacagcaaaatgcacaagtactggctggatacctgctccgagatgtaccttgaaaccttgtgattatccagacattaaacatggaggtctatatcatgagaatatgcgtagaccatactttccagtagctgtaggaaaatattactcctattactgtgatgaacattttgagactccgtcaggaagttactgggatcacattcattgcacacaagatggatggtcgccagcagtaccatgcctcagaaaatgttattttccttatttggaaaatggatataatcaaaatcatggaagaaagtttgtacagggtaaatctatagacgttgcctgccatcctggctacgctcttccaaaagcgcagaccacagttacatgtatggagaatggctggtctcctactcccagatgcatccgtgtcagctttaccctctga

SEQ ID NO: 7 - protein, 2039 aa, synthetic construct
MGASSPRSPEPVGPPAPGLPFCCGGSLLAVVVLLALPVAWGQCNAPEWLPFARPTNLTDEFEFPIGTYLNYECRPGYSGRPFSIICLKNSVWTGAKDRCRRKSCRNPPDPVNGMVHVIKGIQFGSQIKYSCTKGYRLIGSSSATCIISGDTVIWDNETPICDRIPCGLPPTITNGDFISTNRENFHYGSVVTYRCNPGSGGRKVFELVGEPSIYCTSNDDQVGIWSGPAPQCIIPNKCTPPNVENGILVSDNRSLFSLNEVVEFRCQPGFVMKGPRRVKCQALNKWEPELPSCSRVCQPPPDVLHAERTQRDKDNFSPGQEVFYSCEPGYDLRGAASMRCTPQGDWSPAAPTCEVKSCDDFMGQLLNGRVLFPVNLQLGAKVDFVCDEGFQLKGSSASYCVLAGMESLWNSSVPVCEQIFCPSPPVIPNGRHTGKPLEVFPFGKTVNYTCDPHPDRGTSFDLIGESTIRCTSDPQGNGVWSSPAPRCGILGHCQAPDHFLFAKLKTQTNASDFPIGTSLKYECRPEYYGRPFSITCLDNLVWSSPKDVCKRKSCKTPPDPVNGMVHVITDIQVGSRINYSCTTGHRLIGHSSAECILSGNAAHWSTKPPICQRIPCGLPPTIANGDFISTNRENFHYGSVVTYRCNPGSGGRKVFELVGEPSIYCTSNDDQVGIWSGPAPQCIIPNKCTPPNVENGILVSDNRSLFSLNEVVEFRCQPGFVMKGPRRVKCQALNKWEPELPSCSRVCQPPPDVLHAERTQRDKDNFSPGQEVFYSCEPGYDLRGAASMRCTPQGDWSPAAPTCEVKSCDDFMGQLLNGRVLFPVNLQLGAKVDFVCDEGFQLKGSSASYCVLAGMESLWNSSVPVCEQIFCPSPPVIPNGRHTGKPLEVFPFGKAVNYTCDPHPDRGTSFDLIGESTIRCTSDPQGNGVWSSPAPRCGILGHCQAPDHFLFAKLKTQTNASDFPIGTSLKYECRPEYYGRPFSITCLDNLVWSSPKDVCKRKSCKTPPDPVNGMVHVITDIQVGSRINYSCTTGHRLIGHSSAECILSGNTAHWSTKPPICQRIPCGLPPTIANGDFISTNRENFHYGSVVTYRCNLGSRGRKVFELVGEPSIYCTSNDDQVGIWSGPAPQCIIPNKCTPPNVENGILVSDNRSLFSLNEVVEFRCQPGFVMKGPRRVKCQALNKWEPELPSCSRVCQPPPEILHGEHTPSHQDNFSPGQEVFYSCEPGYDLRGAASLHCTPQGDWSPEAPRCAVKSCDDFLGQLPHGRVLFPLNLQLGAKVSFVCDEGFRLKGSSVSHCVLVGMRSLWNNSVPVCEHIFCPNPPAILNGRHTGTPSGDIPYGKEISYTCDPHPDRGMTFNLIGESTIRCTSDPHGNGVWSSPAPRCELSVRAGHCKTPEQFPFASPTIPINDFEFPVGTSLNYECRPGYFGKMFSISCLENLVWSSVEDNCRRKSCGPPPEPFNGMVHINTDTQFGSTVNYSCNEGFRLIGSPSTTCLVSGNNVTWDKKAPICEIISCEPPPTISNGDFYSNNRTSFHNGTVVTYQCHTGPDGEQLFELVGERSIYCTSKDDQVGVWSSPPPRCISTNKCTAPEVENAIRVPGNRSFFTLTEIIRFRCQPGFVMVGSHTVQCQTNGRWGPKLPHCSRVCQPPPEILHGEHTLSHQDNFSPGQEVFYSCEPSYDLRGAASLHCTPQGDWSPEAPRCTVKSCDDFLGQLPHGRVLLPLNLQLGAKVSFVCDEGFRLKGRSASHCVLAGMKALWNSSVPVCEQIFCPNPPAILNGRHTGTPFGDIPYGKEISYACDTHPDRGMTFNLIGESSIRCTSDPQGNGVWSSPAPRCELSVPAACPHPPKIQNGHYIGGHVSLYLPGMTISYICDPGYLLVGKGFIFCTDQGIWSQLDHYCKEVNCSFPLFMNGISKELEMKKVYHYGDYVTLKCEDGYTLEGSPWSQCQADDRWDPPLAKCTSRTHDALIVGTLSGTIFFILLIIFLSWIILKHRKGNNAHENPKEVAIHLHSQGGSSVHPRTLQTNEENSRVLP

SEQ ID NO: 8 - DNA, 6117 bp, synthetic construct
  source 1..6117: mol_type = other DNA
atgggggcctcttctccaagaagcccggagcctgtcgggccgccggcgcccggtctccccttctgctgcggaggatccctgctggcggttgtggtgctgcttgcgctgccggtggcctggggtcaatgcaatgccccagaatggcttccatttgccaggcctaccaacctaactgatgaatttgagtttcccattgggacatatctgaactatgaatgccgccctggttattccggaagaccgttttctatcatctgcctaaaaaactcagtctggactggtgctaaggacaggtgcagacgtaaatcatgtcgtaatcctccagatcctgtgaatggcatggtgcatgtgatcaaaggcatccagttcggatcccaaattaaatattcttgtactaaaggataccgactcattggttcctcgtctgccacatgcatcatctcaggtgatactgtcatttgggataatgaaacacctatttgtgacagaattccttgtgggctaccccccaccatcaccaatggagatttcattagcaccaacagagagaattttcactatggatcagtggtgacctaccgctgcaatcctggaagcggagggagaaaggtgtttgagcttgtgggtgagccctccatatactgcaccagcaatgacgatcaagtgggcatctggagcggccccgcccctcagtgcattatacctaacaaatgcacgcctccaaatgtggaaaatggaatattggtatctgacaacagaagcttattttccttaaatgaagttgtggagtttaggtgtcagcctggctttgtcatgaaaggaccccgccgtgtgaagtgccaggccctgaacaaatgggagccggagctaccaagctgctccagggtatgtcagccacctccagatgtcctgcatgctgagcgtacccaaagggacaaggacaacttttcacctgggcaggaagtgttctacagctgtgagcccggctacgacctcagaggggctgcgtctatgcgctgcacaccccagggagactggagccctgcagcccccacatgtgaagtgaaatcctgtgatgacttcatgggccaacttcttaatggccgtgtgctatttccagtaaatctccagcttggagcaaaagtggattttgtttgtgatgaaggatttcaattaaaaggcagctctgctagttactgtgtcttggctggaatggaaagcctttggaatagcagtgttccagtgtgtgaacaaatcttttgtccaagtcctccagttattcctaatgggagacacacaggaaaacctctggaagtctttccctttgggaaaacagtaaattacacatgcgacccccacccagacagagggacgagcttcgacctcattggagagagcaccatccgctgcacaagtgaccctcaagggaatggggtttggagcagccctgcccctcgctgtggaattctgggtcactgtcaagccccagatcattttctgtttgccaagttgaaaacccaaaccaatgcatctgactttcccattgggacatctttaaagtacgaatgccgtcctgagtactacgggaggccattctctatcacatgtctagataacctggtctggtcaagtcccaaagatgtctgtaaacgtaaatcatgtaaaactcctccagatccagtgaatggcatggtgcatgtgatcacagacatccaggttggatccagaatcaactattcttgtactacagggcaccgactcattggtcactcatctgctgaatgtatcctctcgggcaatgctgcccattggagcacgaagccgccaatttgtcaacgaattccttgtgggctaccccccaccatcgccaatggagatttcattagcaccaacagagagaattttcactatggatcagtggtgacctaccgctgcaatcctggaagcggagggagaaaggtgtttgagcttgtgggtgagccctccatatactgcaccagcaatgacgatcaagtgggcatctggagcggcccggcccctcagtgcattatacctaacaaatgcacgcctccaaatgtggaaaatggaatattggtatctgacaacagaagcttattttccttaaatgaagttgtggagtttaggtgtcagcctggctttgtcatgaaaggaccccgccgtgtgaagtgccaggccctgaacaaatgggagccggagctaccaagctgctccagggtatgtcagccacctccagatgtcctgcatgctgagcgtacccaaagggacaaggacaacttttcacccgggcaggaagtgttctacagctgtgagcccggctatgacctcagaggggctgcgtctatgcgctgcacaccccagggagactggagccctgcagcccccacatgtgaagtgaaatcctgtgatgacttcatgggccaacttcttaatggccgtgtgctatttccagtaaatctccagcttggagcaaaagtggattttgtttgtgatgaaggatttcaattaaaaggcagctctgctagttattgtgtcttggctggaatggaaagcctttggaatagcagtgttccagtgtgtgaacaaatcttttgtccaagtcctccagttattcctaatgggagacacacaggaaaacctctggaagtctttccctttggaaaagcagtaaattacacatgcgacccccacccagacagagggacgagcttcgacctcattggagagagcaccatccgctgcacaagtgaccctcaagggaatggggtttggagcagccctgcccctcgctgtggaattctgggtcactgtcaagccccagatcattttctgtttgccaagttgaaaacccaaaccaatgcatctgactttcccattgggacatctttaaagtacgaatgccgtcctgagtactacgggaggccattctctatcacatgtctagataacctggtctggtcaagtcccaaagatgtctgtaaacgtaaatcatgtaaaactcctccagatccagtgaatggcatggtgcatgtgatcacagacatccaggttggatccagaatcaactattcttgtactacagggcaccgactcattggtcactcatctgctgaatgtatcctctcaggcaatactgcccattggagcacgaagccgccaatttgtcaacgaattccttgtgggctacccccaaccatcgccaatggagatttcattagcaccaacagagagaattttcactatggatcagtggtgacctaccgctgcaatcttggaagcagagggagaaaggtgtttgagcttgtgggtgagccctccatatactgcaccagcaatgacgatcaagtgggcatctggagcggccccgcccctcagtgcattatacctaacaaatgcacgcctccaaatgtggaaaatggaatattggtatctgacaacagaagcttattttccttaaatgaagttgtggagtttaggtgtcagcctggctttgtcatgaaaggaccccgccgtgtgaagtgccaggccctgaacaaatgggagccagagttaccaagctgctccagggtgtgtcagccgcctccagaaatcctgcatggtgagcataccccaagccatcaggacaacttttcacctgggcaggaagtgttctacagctgtgagcctggctatgacctcagaggggctgcgtctctgcactgcacaccccagggagactggagccctgaagccccgagatgtgcagtgaaatcctgtgatgacttcttgggtcaactccctcatggccgtgtgctatttccacttaatctccagcttggggcaaaggtgtcctttgtctgtgatgaagggtttcgcttaaagggcagttccgttagtcattgtgtcttggttggaatgagaagcctttggaataacagtgttcctgtgtgtgaacatatcttttgtccaaatcctccagctatccttaatgggagacacacaggaactccctctggagatattccctatggaaaagaaatatcttacacatgtgacccccacccagacagagggatgaccttcaacctcattggggagagcaccatccgctgcacaagtgaccctcatgggaatggggtttggagcagccctgcccctcgctgtgaactttctgttcgtgctggtcactgtaaaaccccagagcagtttccatttgccagtcctacgatcccaattaatgactttgagtttccagtcgggacatctttgaattatgaatgccgtcctgggtattttgggaaaatgttctctatctcctgcctagaaaacttggtctggtcaagtgttgaagacaactgtagacgaaaatcatgtggacctccaccagaacccttcaatggaatggtgcatataaacacagatacacagtttggatcaacagttaattattcttgtaatgaagggtttcgactcattggttccccatctactacttgtctcgtctcaggcaataatgtcacatgggataagaaggcacctatttgtgagatcatatcttgtgagccacctccaaccatatccaatggagacttctacagcaacaatagaacatcttttcacaatggaacggtggtaacttaccagtgccacactggaccagatggagaacagctgtttgagcttgtgggagaacggtcaatatattgcaccagcaaagatgatcaagttggtgtttggagcagccctccccctcggtgtatttctactaataaatgcacagctccagaagttgaaaatgcaattagagtaccaggaaacaggagtttctttaccctcactgagatcatcagatttagatgtcagcccgggtttgtcatggtagggtcccacactgtgcagtgccagaccaatggcagatgggggcccaagctgccacactgctccagggtgtgtcagccgcctccagaaatcctgcatggtgagcataccctaagccatcaggacaacttttcacctgggcaggaagtgttctacagctgtgagcccagctatgacctcagaggggctgcgtctctgcactgcacgccccagggagactggagccctgaagcccctagatgtacagtgaaatcctgtgatgacttcctgggccaactccctcatggccgtgtgctacttccacttaatctccagcttggggcaaaggtgtcctttgtttgcgatgaagggttccgattaaaaggcaggtctgctagtcattgtgtcttggctggaatgaaagccctttggaatagcagtgttccagtgtgtgaacaaatcttttgtccaaatcctccagctatccttaatgggagacacacaggaactccctttggagatattccctatggaaaagaaatatcttacgcatgcgacacccacccagacagagggatgaccttcaacctcattggggagagctccatccgctgcacaagtgaccctcaagggaatggggtttggagcagccctgcccctcgctgtgaactttctgttcctgctgcctgcccacatccacccaagatccaaaacgggcattacattggaggacacgtatctctatatcttcctgggatgacaatcagctacatttgtgaccccggctacctgttagtgggaaagggcttcattttctgtacagaccagggaatctggagccaattggatcattattgcaaagaagtaaattgtagcttcccactgtttatgaatggaatctcgaaggagttagaaatgaaaaaagtatatcactatggagattatgtgactttgaagtgtgaagatgggtatactctggaaggcagtccctggagccagtgccaggcggatgacagatgggaccctcctctggccaaatgtacctctcgtacacatgatgctctcatagttggcactttatctggtacgatcttctttattttactcatcattttcctctcttggataattctaaagcacagaaaaggcaataatgcacatgaaaaccctaaagaagtggctatccatttacattctcaaggaggcagcagcgttcatccccgaactctgcaaacaaatgaagaaaatagcagggtccttcct

SEQ ID NO: 9 - protein, 62 aa, synthetic construct
KSCPNPGEIRNGQIDVPGGILFGATISFSCNTGYKLFGSTSSFCLISGSSVQWSDPLPECRE

SEQ ID NO: 10 - protein, 63 aa, synthetic construct
IYCPAPPQIDNGIIQGERDHYGYRQSVTYACNKGFTMIGEHSIYCTVNNDEGEWSGPPPECRG

SEQ ID NO: 11 - protein, 65 aa, synthetic construct
IYCPAPPQIDNGIIQGERDHYGYRQSVTYACNKGFTMIGEHSIYCTVNNDEGEWSGPPPECRGKS

SEQ ID NO: 12 - protein, 125 aa, synthetic construct
KSCPNPGEIRNGQIDVPGGILFGATISFSCNTGYKLFGSTSSFCLISGSSVQWSDPLPECREIYCPAPPQIDNGIIQGERDHYGYRQSVTYACNKGFTMIGEHSIYCTVNNDEGEWSGPPPECRG

SEQ ID NO: 13 - protein, 127 aa, synthetic construct
KSCPNPGEIRNGQIDVPGGILFGATISFSCNTGYKLFGSTSSFCLISGSSVQWSDPLPECREIYCPAPPQIDNGIIQGERDHYGYRQSVTYACNKGFTMIGEHSIYCTVNNDEGEWSGPPPECRGKS

SEQ ID NO: 14 - protein, 64 aa, synthetic construct
EDCNELPPRRNTEILTGSWSDQTYPEGTQAIYKCRPGYRSLGNVIMVCRKGEWVALNPLRKCQK

SEQ ID NO: 15 - protein, 64 aa, synthetic construct
EDCNELPPRRNTEILTGSWSDQTYPEGTQAIYKCRPGYRSLGNIIMVCRKGEWVALNPLRKCQK

SEQ ID NO: 16 - protein, 61 aa, synthetic construct
RPCGHPGDTPFGTFTLTGGNVFEYGVKAVYTCNEGYQLLGEINYRECDTDGWTNDIPICEV

SEQ ID NO: 17 - protein, 61 aa, synthetic construct
RPCGHPGDTPFGTFTLTGGNVFEYGVKAVYTCNTGYKLLGEINYRECDTDGWTNDIPICEE

SEQ ID NO: 18 - protein, 61 aa, synthetic construct
GHCQAPDHFLFAKLKTQTNASDFPIGTSLKYECRPEYYGRPFSITCLDNLVWSSPKDVCKR

SEQ ID NO: 19 - protein, 7 aa, synthetic construct
GHHHHHH

SEQ ID NO: 20 - protein, 19 aa, synthetic construct
MGWSCIILFLVATATGVHS

SEQ ID NO: 21 - protein, 188 aa, synthetic construct
EDCNELPPRRNTEILTGSWSDQTYPEGTQAIYKCRPGYRSLGNVIMVCRKGEWVALNPLRKCQKRPCGHPGDTPFGTFTLTGGNVFEYGVKAVYTCNEGYQLLGEINYRECDTDGWTNDIPICEVIYCPAPPQIDNGIIQGERDHYGYRQSVTYACNKGFTMIGEHSIYCTVNNDEGEWSGPPPECRG

SEQ ID NO: 22 - protein, 188 aa, synthetic construct
EDCNELPPRRNTEILTGSWSDQTYPEGTQAIYKCRPGYRSLGNIIMVCRKGEWVALNPLRKCQKRPCGHPGDTPFGTFTLTGGNVFEYGVKAVYTCNEGYQLLGEINYRECDTDGWTNDIPICEVIYCPAPPQIDNGIIQGERDHYGYRQSVTYACNKGFTMIGEHSIYCTVNNDEGEWSGPPPECRG

SEQ ID NO: 23 - protein, 188 aa, synthetic construct
EDCNELPPRRNTEILTGSWSDQTYPEGTQAIYKCRPGYRSLGNVIMVCRKGEWVALNPLRKCQKRPCGHPGDTPFGTFTLTGGNVFEYGVKAVYTCNTGYKLLGEINYRECDTDGWTNDIPICEEIYCPAPPQIDNGIIQGERDHYGYRQSVTYACNKGFTMIGEHSIYCTVNNDEGEWSGPPPECRG

SEQ ID NO: 24 - protein, 188 aa, synthetic construct
EDCNELPPRRNTEILTGSWSDQTYPEGTQAIYKCRPGYRSLGNIIMVCRKGEWVALNPLRKCQKRPCGHPGDTPFGTFTLTGGNVFEYGVKAVYTCNTGYKLLGEINYRECDTDGWTNDIPICEEIYCPAPPQIDNGIIQGERDHYGYRQSVTYACNKGFTMIGEHSIYCTVNNDEGEWSGPPPECRG

SEQ ID NO: 25 - protein, 197 aa, synthetic construct
EDCNELPPRRNTEILTGSWSDQTYPEGTQAIYKCRPGYRSLGNVIMVCRKGEWVALNPLRKCQKRPCGHPGDTPFGTFTLTGGNVFEYGVKAVYTCNEGYQLLGEINYRECDTDGWTNDIPICEVIYCPAPPQIDNGIIQGERDHYGYRQSVTYACNKGFTMIGEHSIYCTVNNDEGEWSGPPPECRGKSGHHHHHH

SEQ ID NO: 26 - protein, 197 aa, synthetic construct
EDCNELPPRRNTEILTGSWSDQTYPEGTQAIYKCRPGYRSLGNIIMVCRKGEWVALNPLRKCQKRPCGHPGDTPFGTFTLTGGNVFEYGVKAVYTCNEGYQLLGEINYRECDTDGWTNDIPICEVIYCPAPPQIDNGIIQGERDHYGYRQSVTYACNKGFTMIGEHSIYCTVNNDEGEWSGPPPECRGKSGHHHHHH

SEQ ID NO: 27 - protein, 197 aa, synthetic construct
EDCNELPPRRNTEILTGSWSDQTYPEGTQAIYKCRPGYRSLGNVIMVCRKGEWVALNPLRKCQKRPCGHPGDTPFGTFTLTGGNVFEYGVKAVYTCNTGYKLLGEINYRECDTDGWTNDIPICEEIYCPAPPQIDNGIIQGERDHYGYRQSVTYACNKGFTMIGEHSIYCTVNNDEGEWSGPPPECRGKSGHHHHHH

SEQ ID NO: 28 - protein, 197 aa, synthetic construct
EDCNELPPRRNTEILTGSWSDQTYPEGTQAIYKCRPGYRSLGNIIMVCRKGEWVALNPLRKCQKRPCGHPGDTPFGTFTLTGGNVFEYGVKAVYTCNTGYKLLGEINYRECDTDGWTNDIPICEEIYCPAPPQIDNGIIQGERDHYGYRQSVTYACNKGFTMIGEHSIYCTVNNDEGEWSGPPPECRGKSGHHHHHH

SEQ ID NO: 29 - protein, 186 aa, synthetic construct
GHCQAPDHFLFAKLKTQTNASDFPIGTSLKYECRPEYYGRPFSITCLDNLVWSSPKDVCKRKSCPNPGEIRNGQIDVPGGILFGATISFSCNTGYKLFGSTSSFCLISGSSVQWSDPLPECREIYCPAPPQIDNGIIQGERDHYGYRQSVTYACNKGFTMIGEHSIYCTVNNDEGEWSGPPPECRG

SEQ ID NO: 30 - protein, 195 aa, synthetic construct
GHCQAPDHFLFAKLKTQTNASDFPIGTSLKYECRPEYYGRPFSITCLDNLVWSSPKDVCKRKSCPNPGEIRNGQIDVPGGILFGATISFSCNTGYKLFGSTSSFCLISGSSVQWSDPLPECREIYCPAPPQIDNGIIQGERDHYGYRQSVTYACNKGFTMIGEHSIYCTVNNDEGEWSGPPPECRGKSGHHHHHH

SEQ ID NO: 31 - protein, 125 aa, synthetic construct
EDCNELPPRRNTEILTGSWSDQTYPEGTQAIYKCRPGYRSLGNVIMVCRKGEWVALNPLRKCQKRPCGHPGDTPFGTFTLTGGNVFEYGVKAVYTCNEGYQLLGEINYRECDTDGWTNDIPICEV

SEQ ID NO: 32 - protein, 125 aa, synthetic construct
EDCNELPPRRNTEILTGSWSDQTYPEGTQAIYKCRPGYRSLGNIIMVCRKGEWVALNPLRKCQKRPCGHPGDTPFGTFTLTGGNVFEYGVKAVYTCNEGYQLLGEINYRECDTDGWTNDIPICEV

SEQ ID NO: 33 - protein, 125 aa, synthetic construct
EDCNELPPRRNTEILTGSWSDQTYPEGTQAIYKCRPGYRSLGNVIMVCRKGEWVALNPLRKCQKRPCGHPGDTPFGTFTLTGGNVFEYGVKAVYTCNTGYKLLGEINYRECDTDGWTNDIPICEE

SEQ ID NO: 34 - protein, 125 aa, synthetic construct
EDCNELPPRRNTEILTGSWSDQTYPEGTQAIYKCRPGYRSLGNIIMVCRKGEWVALNPLRKCQKRPCGHPGDTPFGTFTLTGGNVFEYGVKAVYTCNTGYKLLGEINYRECDTDGWTNDIPICEE

SEQ ID NO: 35 - protein, 199 aa, synthetic construct
QCNAPEWLPFARPTNLTDEFEFPIGTYLKYECRPGYYGRPFSIICLKNSVWTGAKDRCRRKSCRNPPDPVNGMVHVIKDIQFGSQIKYSCTKGYRLIGSSSATCIISGNTVIWDNETPICDRIPCGLPPTITNGDFISTNRENFHYGSVVTYRCNPGSGGRKVFELVGEPSIYCTSNDDQVGIWSGPAPQCIGHHHHHH

SEQ ID NO: 36 - protein, 196 aa, synthetic construct
SCEVPTRLNSASLKQPYITQNYFPVGTVVEYECRPGYRREPSLSPKLTCLQNLKWSTAVEFCKKKSCPNPGEIRNGQIDVPGGILFGATISFSCNTGYKLFGSTSSFCLISGSSVQWSDPLPECREIYCPAPPQIDNGIIQGERDHYGYRQSVTYACNKGFTMIGEHSIYCTVNNDEGEWSGPPPECRGGHHHHHH

SEQ ID NO: 37 - protein, 313 aa, synthetic construct
EDCNELPPRRNTEILTGSWSDQTYPEGTQAIYKCRPGYRSLGNIIMVCRKGEWVALNPLRKCQKRPCGHPGDTPFGTFTLTGGNVFEYGVKAVYTCNEGYQLLGEINYRECDTDGWTNDIPICEVVKCLPVTAPENGKIVSSAMEPDREYHFGQAVRFVCNSGYKIEGDEEMHCSDDGFWSKEKPKCVEISCKSPDVINGSPISQKIIYKENERFQYKCNMGYEYSERGDAVCTESGWRPLPSCEEKSCDNPYIPNGDYSPLRIKHRTGDEITYQCRNGFYPATRGNTAKCTSTGWIPAPRCTLKPGHHHHHH

SEQ ID NO: 38 - protein, 197 aa, synthetic construct; identical to SEQ ID NO: 28

SEQ ID NO: 39 - protein, 193 aa, synthetic construct
GHCQAPDHFLFAKLKTQTNASDFPIGTSLKYECRPEYYGRPFSITCLDNLVWSSPKDVCKRKSCPNPGEIRNGQIDVPGGILFGATISFSCNTGYKLFGSTSSFCLISGSSVQWSDPLPECREIYCPAPPQIDNGIIQGERDHYGYRQSVTYACNKGFTMIGEHSIYCTVNNDEGEWSGPPPECRGGHHHHHH

SEQ ID NO: 40 - protein, 198 aa, synthetic construct
EDCNELPPRRNTEILTGSWSDQTYPEGTQAIYKCRPGYRSLGNIIMVCRKGEWVALNPLRKCQKRPCGHPGDTPFGTFTLTGGNVFEYGVKAVYTCNEGYQLLGEINYRECDTDGWTNDIPICEVVKCLPVTAPENGKIVSSAMEPDREYHFGQAVRFVCNSGYKIEGDEEMHCSDDGFWSKEKPKCVEISGHHHHHH

SEQ ID NO: 41 - protein, 260 aa, synthetic construct
DCGLPPDVPNAQPALEGRTSFPEDTVITYKCEESFVKIPGEKDSVICLKGSQWSDIEEFCNRSCEVPTRLNSASLKQPYITQNYFPVGTVVEYECRPGYRREPSLSPKLTCLQNLKWSTAVEFCKKKSCPNPGEIRNGQIDVPGGILFGATISFSCNTGYKLFGSTSSFCLISGSSVQWSDPLPECREIYCPAPPQIDNGIIQGERDHYGYRQSVTYACNKGFTMIGEHSIYCTVNNDEGEWSGPPPECRGKSGHHHHHH